European Patent Application EP 4 807 004 A1, published September 16, 2026. Title: Reporter cell for measuring TSH activity. Applicant: Cosmic Corporation Co., Ltd. Application JP. The sequence listing filed with the application follows.

SEQUENCE LISTING (5 sequences)

SEQ ID NO: 1 - protein, 92 aa, Homo sapiens
APDVQDCPECTLQENPFFSQPGAPILQCMGCCFSRAYPTPLRSKKTMLVQKNVTSESTCCVAKSYNRVTVMGGFKVENHTACHCSTCYYHKS

SEQ ID NO: 2 - protein, 112 aa, Homo sapiens
FCIPTEYTMHIERRECAYCLTINTTICAGYCMTRDINGKLFLPKYALSQDVCTYRDFIYRTVEIPGCPLHVAPYFSYPVALSCKCGKCNTDYSDCIHEAIKTNYCTKPQKSY

SEQ ID NO: 3 - protein, 764 aa, Homo sapiens
MRPADLLQLVLLLDLPRDLGGMGCSSPPCECHQEEDFRVTCKDIQRIPSLPPSTQTLKLIETHLRTIPSHAFSNLPNISRIYVSIDVTLQQLESHSFYNLSKVTHIEIRNTRNLTYIDPDALKELPLLKFLGIFNTGLKMFPDLTKVYSTDIFFILEITDNPYMTSIPVNAFQGLCNETLTLKLYNNGFTSVQGYAFNGTKLDAVYLNKNKYLTVIDKDAFGGVYSGPSLLDVSQTSVTALPSKGLEHLKELIARNTWTLKKLPLSLSFLHLTRADLSYPSHCCAFKNQKKIRGILESLMCNESSMQSLRQRKSVNALNSPLHQEYEENLGDSIVGYKEKSKFQDTHNNAHYYVFFEEQEDEIIGFGQELKNPQEETLQAFDSHYDYTICGDSEDMVCTPKSDEFNPCEDIMGYKFLRIVVWFVSLLALLGNVFVLLILLTSHYKLNVPRFLMCNLAFADFCMGMYLLLIASVDLYTHSEYYNHAIDWQTGPGCNTAGFFTVFASELSVYTLTVITLERWYAITFAMRLDRKIRLRHACAIMVGGWVCCFLLALLPLVGISSYAKVSICLPMDTETPLALAYIVFVLTLNIVAFVIVCCCYVKIYITVRNPQYNPGDKDTKIAKRMAVLIFTDFICMAPISFYALSAILNKPLITVSNSKILLVLFYPLNSCANPFLYAIFTKAFQRDVFILLSKFGICKRQAQAYRGQRVPPKNSTDIQVQKVTHDMRQGLHNMEDVYELIENSHLTPKKQGQISEEYMQTVL

SEQ ID NO: 4 - DNA, 2295 bp, Homo sapiens
  source 1..2295: mol_type = unassigned DNA
atgaggccggcggacttgctgcagctggtgctgctgctcgacctgcccagggacctgggcggaatggggtgttcgtctccaccctgcgagtgccatcaggaggaggacttcagagtcacctgcaaggatattcaacgcatccccagcttaccgcccagtacgcagactctgaagcttattgagactcacctgagaactattccaagtcatgcattttctaatctgcccaatatttccagaatctacgtatctatagatgtgactctgcagcagctggaatcacactccttctacaatttgagtaaagtgactcacatagaaattcggaataccaggaacttaacttacatagaccctgatgccctcaaagagctccccctcctaaagttccttggcattttcaacactggacttaaaatgttccctgacctgaccaaagtttattccactgatatattctttatacttgaaattacagacaacccttacatgacgtcaatccctgtgaatgcttttcagggactatgcaatgaaaccttgacactgaagctgtacaacaatggctttacttcagtccaaggatatgctttcaatgggacaaagctggatgctgtttacctaaacaagaataaatacctgacagttattgacaaagatgcatttggaggagtatacagtggaccaagcttgctggacgtgtctcaaaccagtgtcactgcccttccatccaaaggcctggagcacctgaaggaactgatagcaagaaacacctggactcttaagaaacttccactttccttgagtttccttcacctcacacgggctgacctttcttacccaagccactgctgtgcttttaagaatcagaagaaaatcagaggaatccttgagtccttgatgtgtaatgagagcagtatgcagagcttgcgccagagaaaatctgtgaatgccttgaatagccccctccaccaggaatatgaagagaatctgggtgacagcattgttgggtacaaggaaaagtccaagttccaggatactcataacaacgctcattattacgtcttctttgaagaacaagaggatgagatcattggttttggccaggagctcaaaaacccccaggaagagactctacaagcttttgacagccattatgactacaccatatgtggggacagtgaagacatggtgtgtacccccaagtccgatgagttcaacccgtgtgaagacataatgggctacaagttcctgagaattgtggtgtggttcgttagtctgctggctctcctgggcaatgtctttgtcctgcttattctcctcaccagccactacaaactgaacgtcccccgctttctcatgtgcaacctggcctttgcggatttctgcatggggatgtacctgctcctcatcgcctctgtagacctctacactcactctgagtactacaaccatgccatcgactggcagacaggccctgggtgcaacacggctggtttcttcactgtctttgcaagcgagttatcggtgtatacgctgacggtcatcaccctggagcgctggtatgccatcaccttcgccatgcgcctggaccggaagatccgcctcaggcacgcatgtgccatcatggttgggggctgggtttgctgcttccttctcgccctgcttcctttggtgggaataagtagctatgccaaagtcagtatctgcctgcccatggacaccgagacccctcttgctctggcatatattgtttttgttctgacgctcaacatagttgccttcgtcatcgtctgctgctgtcatgtgaagatctacatcacagtccgaaatccgcagtacaacccaggggacaaagataccaaaattgccaagaggatggctgtgttgatcttcaccgacttcatatgcatggccccaatctcattctatgctctgtcagcaattctgaacaagcctctcatcactgttagcaactccaaaatcttgctggtactcttctatccacttaactcctgtgccaatccattcctctatgctattttcaccaaggccttccagagggatgtgttcatcctactcagcaagtttggcatctgtaaacgccaggctcaggcataccgggggcagagggttcctccaaagaacagcactgatattcaggttcaaaaggttacccacgacatgaggcagggtctccacaacatggaagatgtctatgaactgattgaaaactcccatctaaccccaaagaagcaaggccaaatctcagaagagtatatgcaaacggttttgtaa

SEQ ID NO: 5 - skipped